European Patent Application EP 4 260 872 A1, published October 18, 2023. Title: Agent for preventing or treating frontotemporal lobar degeneration. Applicant: NATIONAL UNIVERSITY CORPORATION TOKYO MEDICAL AND DENTAL UNIVERSITY. The sequence listing filed with the application follows.

SEQUENCE LISTING (16 sequences)

SEQ ID NO: 1 - protein, 5 aa, Artificial
  Heavy Chain Complementarity Determination Region 1 of human monoc lonal antibody #129
  MISC_FEATURE: Inventor:OKAZAWA, Hitoshi
SYAMS

SEQ ID NO: 2 - protein, 17 aa, Artificial
  Heavy Chain Complementarity Determination Region 2 of human monoc lonal antibody #129
DISGSGGSTYYADSVKG

SEQ ID NO: 3 - protein, 6 aa, Artificial
  Heavy Chain Complementarity Determination Region 3 of human monoc lonal antibody #129
GYGMDV

SEQ ID NO: 4 - protein, 11 aa, Artificial
  Light Chain Complementarity Determination Region 1 of human monoc lonal antibody #129
RASQSVTNYLA

SEQ ID NO: 5 - protein, 7 aa, Artificial
  Light Chain Complementarity Determination Region 2 of human monoc lonal antibody #129
GASILET

SEQ ID NO: 6 - protein, 9 aa, Artificial
  Light Chain Complementarity Determination Region 3 of human monoc lonal antibody #129
LQHNSTPLT

SEQ ID NO: 7 - protein, 115 aa, Artificial
  Heavy Chain Variable Region of human monoclonal antibody #129
EVQLLESGGGLVQPGGSLRLSCAASGFTFSSYAMSWVRQAPGKGLEWVSDISGSGGSTYYADSVKGRFTISRDNSKNTLYLQMNSLRAEDTAVYYCARGYGMDVWGQGTMVTVSS

SEQ ID NO: 8 - protein, 107 aa, Artificial
  Light Chain Variable Region of human monoclonal antibody #129
DIQMTQSPSSLSASVGDRVTITCRASQSVTNYLAWYQQKPGKAPKLLIYGASILETGVPSRFSGSGSGTDFTLTINSLQPEDFATYYCLQHNSTPLTFGQGTKLEIK

SEQ ID NO: 9 - protein, 445 aa, Artificial
  Heavy Chain of human monoclonal antibody #129
EVQLLESGGGLVQPGGSLRLSCAASGFTFSSYAMSWVRQAPGKGLEWVSDISGSGGSTYYADSVKGRFTISRDNSKNTLYLQMNSLRAEDTAVYYCARGYGMDVWGQGTMVTVSSASTKGPSVFPLAPSSKSTSGGTAALGCLVKDYFPEPVTVSWNSGALTSGVHTFPAVLQSSGLYSLSSVVTVPSSSLGTQTYICNVNHKPSNTKVDKKVEPKSCDKTHTCPPCPAPELLGGPSVFLFPPKPKDTLMISRTPEVTCVVVDVSHEDPEVKFNWYVDGVEVHNAKTKPREEQYNSTYRVVSVLTVLHQDWLNGKEYKCKVSNKALPAPIEKTISKAKGQPREPQVYTLPPSREEMTKNQVSLTCLVKGFYPSDIAVEWESNGQPENNYKTTPPVLDSDGSFFLYSKLTVDKSRWQQGNVFSCSVMHEALHNHYTQKSLSLSPGK

SEQ ID NO: 10 - protein, 213 aa, Artificial
  Light Chain of human monoclonal antibody #129
DIQMTQSPSSLSASVGDRVTITCRASQSVTNYLAWYQQKPGKAPKLLIYGASILETGVPSRFSGSGSGTDFTLTINSLQPEDFATYYCLQHNSTPLTFGQGTKLEIKTVAAPSVFIFPPSDEQLKSGTASVVCLLNNFYPREAKVQWKVDNALQSGNSQESVTEQDSKDSTYSLSSTLTLSKADYEKHKVYACEVTHQGLSSPVTKSFNRGEC

SEQ ID NO: 11 - DNA, 25 bp, Artificial
  primer 1
atatgctctcactgtatggtattgc

SEQ ID NO: 12 - DNA, 25 bp, Artificial
  primer 2
tccagatgagcttagaagattagaa

SEQ ID NO: 13 - DNA, 25 bp, Artificial
  primer 3
tggattttatttatgtctgaatgtg

SEQ ID NO: 14 - DNA, 25 bp, Artificial
  primer 4
ataagcaacttcacaaggcatctta

SEQ ID NO: 15 - DNA, 25 bp, Artificial
  primer 5
acagttgggtgtgatagcaggtact

SEQ ID NO: 16 - DNA, 25 bp, Artificial
  primer 6
tcgagaattacaggaatgtatcatc